European Patent Application EP 4 506 468 A1, published February 12, 2025. Title: Method for diagnosing cognitive impairment through adipose tissue / blood and compounds useful for its treatment. Applicant: Fundacio Institut d Investigacio Biomedica de Girona Dr Josep Trueta. The sequence listing filed with the application follows.

SEQUENCE LISTING (49 sequences)

SEQ ID NO: 1 - DNA, 3831 bp, Homo sapiens
  source 1..3831: mol_type = genomic DNA; note = nucleotide sequence of SLC18A2 gene NCBI Ref NM_003054.6; note (original language) = secuencia de nucleotidos del gen SLC18A2 Ref NM_003054.6
ggggcggagactgcgacccggagccgcccggactgacggagcccactgcggtgcgggcgttggcgcgggcacggaggacccgggcaggcatcgcaagcgaccccgagcggagccccggagccatggccctgagcgagctggcgctggtccgctggctgcaggagagccgccgctcgcggaagctcatcctgttcatcgtgttcctggcgctgctgctggacaacatgctgctcactgtcgtggtccccatcatcccaagttatctgtacagcattaagcatgagaagaatgctacagaaatccagacggccaggccagtgcacactgcctccatctcagacagcttccagagcatcttctcctattatgataactcgactatggtcaccgggaatgctaccagagacctgacacttcatcagaccgccacacagcacatggtgaccaacgcgtccgctgttccttccgactgtcccagtgaagacaaagacctcctgaatgaaaacgtgcaagttggtctgttgtttgcctcgaaagccaccgtccagctcatcaccaaccctttcataggactactgaccaacagaattggctatccaattcccatatttgcgggattctgcatcatgtttgtctcaacaattatgtttgccttctccagcagctatgccttcctgctgattgccaggtcgctgcagggcatcggctcgtcctgctcctctgtggctgggatgggcatgcttgccagtgtctacacagatgatgaagagagaggcaacgtcatgggaatcgccttgggaggcctggccatgggggtcttagtgggcccccccttcgggagtgtgctctatgagtttgtggggaagacggctccgttcctggtgctggccgccctggtactcttggatggagctattcagctctttgtgctccagccgtcccgggtgcagccagagagtcagaaggggacacccctaaccacgctgctgaaggacccgtacatcctcattgctgcaggctccatctgctttgcaaacatgggcatcgccatgctggagccagccctgcccatctggatgatggagaccatgtgttcccgaaagtggcagctgggcgttgccttcttgccagctagtatctcttatctcattggaaccaatatttttgggatacttgcacacaaaatggggaggtggctttgtgctcttctgggaatgataattgttggagtcagcattttatgtattccatttgcaaaaaacatttatggactcatagctccgaactttggagttggttttgcaattggaatggtggattcgtcaatgatgcctatcatgggctacctcgtagacctgcggcacgtgtccgtctatgggagtgtgtacgccattgcggatgtggcattttgtatggggtatgctataggtccttctgctggtggtgctattgcaaaggcaattggatttccatggctcatgacaattattgggataattgatattctttttgcccctctctgcttttttcttcgaagtccacctgccaaagaagaaaaaatggctattctcatggatcacaactgccctattaaaacaaaaatgtacactcagaataatatccagtcatatccgataggtgaagatgaagaatctgaaagtgactgagatgagatcctcaaaaatcatcaaagtgtttaattgtataaaacagtgtttccagtgacacaactcatccagaactgtcttagtcataccatccatccctggtgaaagagtaaaaccaaaggttattatttcctttccatggttatggtcgattgccaacagccttataaagaaaaagaagcttttctaggggtttgtataaatagtgttgaaactttattttatgtatttaattttattaaatatcatacaatatattttgatgaaataggtattgtgtaaatctataaatatttgaatccaaaccaaatataattttttaacttacattaacaaacatttgggcaaaaatcatattggtaatgagtgtttaaaattaaagcacacattatctctgagactcttccaacaaagagaaactagaatgaagtctgaaaaacagaatcaagtaagacagcatgttatatagtgacactgaatgttatttaacttgtagttactatcaatatatttatgcgttaaacagctagttctctcaagtgtagaggacaagaacttgtgtcagttatcttttgaatccataaatcttagctggcattagttttctatgtaatcacctacctagagagagttgtaaattatatgttaacatgttatctggttggcagcaaacactaaagccaataaaggaaaaacagtaaatgttccgaaagcagagaaaagcaaccaaacatattgttatgaactaaaagctttccctttaagatgcatacttgtcttactggatgaagaaaattgagggtacatgtaccttatactgtcaaggttgtttaaacatgataaggttaatcgccatctacttcaagttttagaaaaggaaacaagaagctgaaaacagctgctctgactttaatatctgactatatctttgatctgtttgcaggtcatccaagtgttttctaggaatatatttattttaggttgtctgaaactactattttttagactcctgaaagttgttcacatcaatgtgaagacaaattttaaatgaaaatgaagaatgaaattatgtcttgaatcatatattaagaagtaaaaataatagtgatcaggcagaaaagaaaaatggaacatctaaaaatgtatgtgctaactatatcatccagtgtgcagtgttgtgtatttttctaagcatgacaacattgatgtgccttttcagtgtaacagcaaatactgttagtgaacattgtcaatttatgtcattttgttaagagatatgactggagtgtgcagtgtggaatgtctctaatactacttgtgaatcctgcagttctataatcataaacaaaaattacttagtttcgttaagctaagattgtgtttgtgttaacttcgacatcaaggagcaaagaactttagaacagactcctcaatcttgtgactttcttattctctaggaaagtaacacttcgtttcatgaagcttttctgtggggcttcgattatttcaagtctggtttctaagtgcagtgtgtttgaagcaaacgaacttccaactcacttatttggcattgggcaacttggccaagtctgccactttggaagatggctctggaggaaactctcatatggctaaaaaggcaggctagtttcttacttctacaggggtagagccttaaaaaagaacgtgctacaaattggttctctttgagggtttctggttctccctgcccccaataccatatactttattgcaattttatttttgcctttacggctctgtgtctttctgcaagaaggcctggcaaaggtatgcctgctgttggtccctcgggataagataaaatataaataaaaccttcagaactgttttggagcaaaagatagcttgtacttggggaaaaaaattctaagttcttttatatgactaatattcttggttagcaagactggaaagaggtgtttttttaaaatgtacataccagaacaaagaacatacagctctctgaacatttattttttgaacagaggtggtttttatgtttggacctggtaatacagatacaaaaactttaatgaggtagcaatgaatattcaactgtttgactgctaagtgtatctgtccatattttagcaagtttacttaataaatcttctgaaccatg

SEQ ID NO: 2 - protein, 514 aa, Homo sapiens
  source 1..514: note = amino acid sequence of SLC18A2 protein NCBI Ref NP_003045.2; note (original language) = secuencia de aminoacidos de la proteina SLC18A2 NCBI Ref NP_003045.2
MALSELALVRWLQESRRSRKLILFIVFLALLLDNMLLTVVVPIIPSYLYSIKHEKNATEIQTARPVHTASISDSFQSIFSYYDNSTMVTGNATRDLTLHQTATQHMVTNASAVPSDCPSEDKDLLNENVQVGLLFASKATVQLITNPFIGLLTNRIGYPIPIFAGFCIMFVSTIMFAFSSSYAFLLIARSLQGIGSSCSSVAGMGMLASVYTDDEERGNVMGIALGGLAMGVLVGPPFGSVLYEFVGKTAPFLVLAALVLLDGAIQLFVLQPSRVQPESQKGTPLTTLLKDPYILIAAGSICFANMGIAMLEPALPIWMMETMCSRKWQLGVAFLPASISYLIGTNIFGILAHKMGRWLCALLGMIIVGVSILCIPFAKNIYGLIAPNFGVGFAIGMVDSSMMPIMGYLVDLRHVSVYGSVYAIADVAFCMGYAIGPSAGGAIAKAIGFPWLMTIIGIIDILFAPLCFFLRSPPAKEEKMAILMDHNCPIKTKMYTQNNIQSYPIGEDEESESD

SEQ ID NO: 3 - DNA, 5700 bp, Homo sapiens
  source 1..5700: mol_type = genomic DNA; note = nucleotide sequence of RIMS1 gene NCBI Ref NM_001168407.2; note (original language) = Secuencia de nucleotidos del gen RIMS1 NCBI Ref NM_001168407.2
gcacagtgcctgcagtgacctgagtcagtcatgcaaggagactttcttgttctcacaccaatgttttatttcagtttccattttctgctggtcctgttgttcaatgatataagcagagtgatgaaggaggcgcttcacactcttcttagataagatcttgagcagcagagagtggtttaaacagcaaggcttaaatctctcaagctggatttatttccaagtttgctgtcatgtgtgcacctgggattcatgtctcttcagaagggtgggaagaagtgaggtctgttgattccgaagagggaacaattgaagctcgacgagcagttgctggtgatttggattattactggttggatcctgccacgtggcacagccgggagacatcacctattagttcgcatcctgtaacgtggcaaccatctaaagagggggaccgattaattggacgtgttattcttaacaagagaacaaccatgcccaaagactcaggtgcattgctgggtctgaaagttgttggaggaaaaatgactgacttaggacgacttggtgctttcatcaccaaagtaaagaagggtagcctagcagatgtagttggacacctaagagcaggggatgaagttctagaatggaatggtaaacccctgccgggagctacaaatgaagaagtttacaacattattttagaatcaaaatcagaacctcaagttgaaattattgtttcaaggcctattggtgacattccccggattcctgagagctcccaccctccactggagtccagttcaagttcctttgaatctcagaagatggaaaggccttccatttctgttatttctccaacaagtcctggagctctaaaagatgccccacaagtcttaccagggcaactttctgtgaagttgtggtatgataaagtgggacaccagctgattgtaaatgttctgcaagcaacagatctacctgctagagtagatggacgtcctcgaaatccctatgtaaaaatgtattttcttccagatagaagtgataaaagtaaaaggaggaccaaaacagtaaagaaaatactagaaccaaaatggaatcaaacttttgtctattcacatgtacatcgtagagattttagagaacgaatgttagaaataactgtgtgggaccaaccaagagtgcaagaagaagaaagtgaatttcttggagagatcctcatagaattggagacagcgcttttagatgatgaaccgcattggtataaacttcagacacatgatgagtcttcactacctctgcctcagccatcacctttcatgccaaggcgacatattcatggagaaagctctagcaaaaagctacaaagatctcagcgaatcagtgatagtgacatctcagattatgaggttgatgatggtattggcgtagttcctccaggctataggtctagtgctagagaaagtaaatctacaacattaactgtgccagaacagcaaagaacaactcatcaccgctcacgttcagtatctcctcatcgcggcaatgatcagggaaagccgcgttcacgtttaccaaatgtgccattacagaggagtttagatgaaattcatccaacaagaaggtcacgttctccaaccagacaccatgatgcctcccgaagtccagttgatcatagaaccagagatgtggatagtcagtatttatcagaacaagacagtgagcttcttatgctgcccagagcaaaacgaggacgaagtgcagaatgcctacatactaccagtgaactgcagccctttcttgacagggctaggagtgctagtaccaactgcttgagaccagatactagtttgcattcaccagaacgagaaaggcactccagaaagtctgaaagatctagcatccaaaaacagactaggaaaggcactgcctctgatgcagaaagaatgcaccgacagagaagtccaacacaatctcctccagcagacacatcgttcagcagtcgcaggggaagacagctcccacaagtgccagtgagaagcggcagtatagaacaagcaagcttagtagtggaggagcgaacaagacagatgaaaatgaaagtgcatcgatttaagcagacaacagggtctggttctagtcaagaacttgatcgcgagcaatattccaagtataacatacataaagatcagtacagaagctgtgataacgtctctgccaaatcatcagatagtgatgtcagtgatgtttccgccatttcccgaaccagcagtgcctcacgcctcagcagcacaagctttatgtcagagcaatctgagcgccccaggggtagaatcagttcatttacccccaaaatgcaaggcagacggatggggacttcaggaagatccatcatgaagagcaccagtgtcagtggagagatgtacacactggagcataatgacggcagccagtcagacacagctgtgggtacagttggagcaggtggaaagaaacggagatccagccttagtgccaaagtggttgccatagtgtctcgaaggagtagaagcacatcccagcttagtcaaacagagtcgggccacaaaaagttaaaaagtaccatccagagaagcacagaaacaggcatggcagctgaaatgagaaagatggtaaggcagccgagccgagagtctactgatggcagcatcaacagttacagctctgagggcaatttaatatttcctggagtgcgactgggagctgacagtcaattcagtgattttcttgatggattgggaccagcccagcttgttggccgccaaacccttgccacccctgcaatgggtgatatacaaataggaatggaggacaaaaagggccaattagaagtggaagtcattagagcacgaagcctcacacaaaagcctggttccaaatctacacctgctccatatgtcaaagtatatcttttggaaaatggggcctgtatagccaagaagaagacaagaattgcacgaaaaacccttgatcctttgtatcagcagtctctggtttttgatgaaagtccacagggtaaagttcttcaggtgattgtctggggagactatggcagaatggaccacaaatgctttatgggtgtggctcagatcttgttggaagaactcgacctgtccagcatggtgatcggatggtacaaattgttcccaccgtcctcactggtggatcccacactcactcccctcacccggcgggcttcccagtcatctctggaaagttcaactgggcctccctgtattcgatcatagtgaactcataccagagtcattccaataaaactctacttttcaggataataatctgaaccagatatttcatgatcgaaagcattgttggagacagacaatcaacttgtgttttgcctgtagtagtttttcaataatatgtcccaattgttatttaaaacatggcttcatatgacagaacaaggcaatctatcaaatttacaggaagaatcaacatgctggtgagagtcactgatgcttctaacaaatagaaaaagaggaaactttaaatccacgcatacacgtacacacacacatgcacacacacacacaccaaattgaacaaactggaaactctcactctgtgaaaagttgtattctacacatttctgcacagaccacaagcagtgttatttccctgatgtttgagttgttttgttcttttgtgtgttttgtttatttgtgtgttgtttgttggttttcgtttcttgagtttttgttttgttttcaccacatctgttatttccactagtttttttttggctgtgtcatgacaggcctcatgatgctaacagagattcttcccttcttttttccaaaagcaccaaaaaaaagggctgaagtagtctctgtagcatctccccaaagtgttaaacagctacataaggtgaagccaaggaagggtttcactagctttcattttataattatttaaagtcttatgtgtggatacccaagagacaaaaagttatcttccaaaataaataatcacagaagtacttttttaatgaagagcctatctgtttgcattctagaaaattaatttatggtttccattgttttgcatggaagacttttaaagaagtcaatctgcaactaatgctggggactaaaactaactgcataattgtactttgaaaacactccttgtaatgcctttttcttcctgatattaaaaaaatgctcatgtgtataaaccatactttgacttcccaaaaatggtgactaggaatggatttgagcctaagacactttgagctatgcccaggcttctcagccatacctcagtgtagacacatccatctgccctggaaagagcatggtatgagctgttcaatattccactggaaattccagttgaaatattctgcactaaactattgtttttattgaattttagtttacatttctttgagattgatgcaagcacaaagcttgattttttaatgcaaagtatcttactttttggggggaaaataaacaaaatgaactttcaatttgcattttcatttagtttctcttggccttgaatttcccttgtgacattctgtacatgtgctacaaactgcagtctctgcaggtgcattgatatgttctccctccttttatgagtcactccacttttgtgattacacaaatagagcagcatgacttggaactgttcagagctgcatgcacattttgtaaaaaaaaaaaattttaaaaagaaaagaaacaaaaggttatttaataatgtatgttagttccacataggccagcttgtatgttgcatgtacttgtacagtttgcttgttaattactataccgaaataaccaagaaatctaagccatccacttttgttatagacattttgcaggttttagccagactcagtctctgggtctgtggtgaaatgtctatagatggactttattttttaccctccggaaaacgtgatgtagtacggaccaaattccttctaataaatattttggtgtagattcctactgtggggctgtaacacatgtagacactgtgtacacactaggttttaattcatagacatactgcctgcaccaagtgaattatttattattatttacacatgccagaattatctgcccatcattccacagggcacagattgaccactgctcaccatgctgagtaggaggaactgaagcattggtgcacttctactagattccgttctgtcttagtggccaacaatcaactgattataattgggtagtatctttctattttgaccacttgtcttaacactcccctgtgcttttaaatgaaattccaattcatgtatgtaaacatgtttaataaaatttacttttcatgtcagtcagtagccatatgtgttctatgtcttgccagatttccattgtgggttctatggtgcaaaatgggagccaggccatgggaaggggaggctggggtttgttgtctgctgcgggcatttgacttgacttgtcactgcactatattatgtcttaatcgatggcccaaagggtactttgcatcacatacaagttttcacttcgtcagcctgtctaagtgagcacatgactatacttctgaaaagtggcattattaaaaataataaatctcagtaagaatcaaatggaaggttgttttctgctgctgtttgaatgtgctaataaaagagacaactctattgtc

SEQ ID NO: 4 - protein, 1012 aa, Homo sapiens
  source 1..1012: note = amino acid sequence of RIMS1 protein NCBI Ref NP_001161879.1; note (original language) = secuencia de aminoacidos de la proteina RIMS1 NCBI Ref NP_001161879.1
MCAPGIHVSSEGWEEVRSVDSEEGTIEARRAVAGDLDYYWLDPATWHSRETSPISSHPVTWQPSKEGDRLIGRVILNKRTTMPKDSGALLGLKVVGGKMTDLGRLGAFITKVKKGSLADVVGHLRAGDEVLEWNGKPLPGATNEEVYNIILESKSEPQVEIIVSRPIGDIPRIPESSHPPLESSSSSFESQKMERPSISVISPTSPGALKDAPQVLPGQLSVKLWYDKVGHQLIVNVLQATDLPARVDGRPRNPYVKMYFLPDRSDKSKRRTKTVKKILEPKWNQTFVYSHVHRRDFRERMLEITVWDQPRVQEEESEFLGEILIELETALLDDEPHWYKLQTHDESSLPLPQPSPFMPRRHIHGESSSKKLQRSQRISDSDISDYEVDDGIGVVPPGYRSSARESKSTTLTVPEQQRTTHHRSRSVSPHRGNDQGKPRSRLPNVPLQRSLDEIHPTRRSRSPTRHHDASRSPVDHRTRDVDSQYLSEQDSELLMLPRAKRGRSAECLHTTSELQPFLDRARSASTNCLRPDTSLHSPERERHSRKSERSSIQKQTRKGTASDAERMHRQRSPTQSPPADTSFSSRRGRQLPQVPVRSGSIEQASLVVEERTRQMKMKVHRFKQTTGSGSSQELDREQYSKYNIHKDQYRSCDNVSAKSSDSDVSDVSAISRTSSASRLSSTSFMSEQSERPRGRISSFTPKMQGRRMGTSGRSIMKSTSVSGEMYTLEHNDGSQSDTAVGTVGAGGKKRRSSLSAKVVAIVSRRSRSTSQLSQTESGHKKLKSTIQRSTETGMAAEMRKMVRQPSRESTDGSINSYSSEGNLIFPGVRLGADSQFSDFLDGLGPAQLVGRQTLATPAMGDIQIGMEDKKGQLEVEVIRARSLTQKPGSKSTPAPYVKVYLLENGACIAKKKTRIARKTLDPLYQQSLVFDESPQGKVLQVIVWGDYGRMDHKCFMGVAQILLEELDLSSMVIGWYKLFPPSSLVDPTLTPLTRRASQSSLESSTGPPCIRS

SEQ ID NO: 5 - DNA, 998 bp, Homo sapiens
  source 1..998: mol_type = genomic DNA; note = nucleotide sequence of NUDT2 gene NCBI Ref NM_001161.5; note (original language) = secuencia de nucleotidos del gen NUDT2 NCBI Ref NM_001161.5
aaggtccgcctcctacctccttctgcttcggggagggcatgggatcagctacctgtttctgcctcaaccacggaccaataatatgagatctttgttcaccagttctacagtgatggggtgcttccttttggcttctggaatgggtgcgtttgcttctgaggatctccagtgtcacaacaaacacatgccagccctgttttacagggagccctggaggagttgggatagaggccacattgactgagggtagttgccagggtcctgcagttatacacaaagtccttaggataagaccatggccttgagagcatgtggcttgatcatcttccgaagatgcctcattcccaaagtggacaacaatgcaattgagtttttactgctgcaggcatcagatggcattcatcactggactcctcccaaaggccatgtggaaccaggagaggatgacttggaaacagccctgagggagacccaagaggaagcaggcatagaagcaggccagctgaccattattgaggggttcaaaagggaactcaattatgtggccaggaacaagcctaaaacagtcatttactggctggcggaggtgaaggactatgacgtggagatccgcctctcccatgagcaccaagcctaccgctggctggggctggaggaggcctgccagttggctcagttcaaggagatgaaggcagcgctccaagaaggacaccagtttctttgctccatagaggcctgagctgactggagcagagtcatttgcttcagcaggatccttgtgggccttctaagatgaagccaccctcaggtccagggaaggttgtgctggtatttggctcatgacagccaagagcagatttgtgaaatcggctcaactcccaggtgagagcaagcaaaaatcttggctgggtggaaaggaaggcaaaagagtaaaaattaaaaaggccaggcccagtaagtgtaccttgtactttataaataaacctcaagcagctcaa

SEQ ID NO: 6 - protein, 147 aa, Homo sapiens
  source 1..147: note = amino acid sequence of NUDT2 protein NCBI Ref NP_001152.1; note (original language) = secuencia de aminoacidos de la proteina NUDT2 NCBI Ref NP_001152.1
MALRACGLIIFRRCLIPKVDNNAIEFLLLQASDGIHHWTPPKGHVEPGEDDLETALRETQEEAGIEAGQLTIIEGFKRELNYVARNKPKTVIYWLAEVKDYDVEIRLSHEHQAYRWLGLEEACQLAQFKEMKAALQEGHQFLCSIEA

SEQ ID NO: 7 - DNA, 3224 bp, Homo sapiens
  source 1..3224: mol_type = genomic DNA; note = nucleotide sequence of AMPH gene NCBI Ref NM_001635.4; note (original language) = secuencia de nucleotidos del gen AMPH NCBI Ref NM_001635.4
gcagctccccggacccgcagccatggccgacatcaagacgggcatcttcgccaagaacgtccagaagcgactcaaccgcgcgcaggaaaaggtcctccaaaagctggggaaagctgatgagacaaaagacgaacagttcgaagaatatgtccagaacttcaaacggcaagaagcagagggtaccagacttcagcgagaactccgaggatatttagcagcaatcaaaggcatgcaggaggcctccatgaagctcacagagtcgctgcatgaagtctatgagcctgactggtatgggcgggaagatgtgaaaatggttggtgagaaatgtgatgtgctgtgggaagacttccatcaaaaactcgtggatgggtccttgctaacactggatacctacctggggcaatttcctgacataaagaatcgcatcgccaagcgcagcaggaagctagtggactatgacagtgcccgccaccatctggaagctctgcagagctccaagaggaaggatgagagtcgaatctctaaggcagaagaagaatttcagaaagcacagaaagtgtttgaagagtttaacgttgacttacaagaagagttaccatcattatggtcaagacgagttggattttatgttaatactttcaaaaacgtctccagccttgaagccaagtttcataaggaaattgcggtgctttgccacaaactgtatgaagtgatgacaaaactgggtgaccagcacgccgacaaggccttcaccatccaaggagcgcccagtgattcgggtcctctccgcattgcaaagacaccatcaccgcctgaggagccttcacccctcccgagcccgacagcaagtccaaatcatacattagcacctgcgtctcccgcaccagcacggcctcggtcaccttcacagacaaggaaagggcctcctgtcccacctctacctaaagtcaccccgacaaaggaactgcagcaggagaacatcatcagtttctttgaggacaactttgttccagaaatcagtgtgacaacaccttcccagaatgaagtccctgaggtgaagaaagaggagactttgctggatctggactttgatcctttcaagcccgaggtgacacctgcaggttctgctggagtgacccactcacccatgtctcagacattgccctgggacctatggacgacaagcactgatttggtacagccggcttctggtggttcatttaatggattcacacagccccaggatacttcattattcacaatgcagacagaccagagtatgatctgcaacttggctgaatctgaacaggctccacccacagagccaaaagcagaggagcctctggctgctgtcacacctgccgttggtctggaccttggaatggacactcgggctgaggagccagtggaggaggcagtgatcatacctggagctgatgctgatgcagctgttggaaccttggtgtcagcagctgagggggccccaggagaggaagcagaggcggagaaggccactgtccctgccggggaaggagtaagtttagaggaggccaaaattggaactgaaaccactgagggtgcagagagtgcccaacctgaagcagaggagctcgaagcaacagtgcctcaggagaaggtcattccttcggtggtcatagagcctgcctccaaccatgaagaggaaggagaaaacgaaataactataggtgcagagcccaaggagaccaccgaggacgcggctcctccgggccccaccagcgagacaccggagctggctacggagcagaagcctatccaggaccctcagcccacgccttctgcaccagccatgggggctgctgaccagctagcatctgcaagggaggcctctcaggaattgcctcctggctttctctacaaggtggaaacactgcatgattttgaggcagcaaattctgatgaacttaccttacaaaggggtgatgtggtgctggtggtcccctcagattcagaagctgatcaggatgcaggctggctggtgggagtgaaggaatcagactggcttcagtacagagaccttgccacctacaaaggcctctttccagagaacttcacccgacgcttagattagggcaacaagtactgcaagaaggagctcagttacggggtttttaaaccttcatgaaaacctgaagagttcacttttgttattatgctcttaatgatttacagactgatgccagacaaaccttgggaagatgtatcaatggagcatgtgtgcaaaaaaatgtaagaggaaaaaaagtaaattaaggaaaaaatcctcactcattcccatgttgtcaataacaggtttgtttgtgctttgtccaagctgtggagactcttgtacttgatcccctcccaccaattctaaagtagctttctccagatcagactttaatttctctgcatcaggtgtatcgtattgagtggctgccctgcagaagatgtgatgaattatcctgtagtacaagattatcttattcccctgcccaggtgtgagcacgtgctctcgctccctttcaggtttactatgtttaaaactaaactgctgcaaaagttctcaatgttcttttccaacacatctatatatatatggacacacagtcacgcaagctagttcccatgactcctggatctatgtgtatgcagaaggctacatatacatagttgcttctttcctttccattgtagctctttgcctctcaattgtcattgatacatgcattgctcttattctgtctggcattacaattgcagttttgcctaatggcaaaaccagccatcccattggcaaaagagtcaacagtatctgtgtttgtactgtgcagttttcaggatgagatgacagatagcacgactacactgaggcaccctcagagaaggcagggcctgatttatctagctgtccagccgctgtggctggaggtaggctagttgggatgggcagctaagcagtcttctcttctgcctttatgagattgggtagaaagatggggcatattcatctacccccaaaagaacactataaaaacagctcctctatatttccacctctttctatttatgcaactcatcttcacagattgttctaaagtaaaatagatggtgtatgctgtatccacaaatcatctgtaacaattatgttttcagtgctgtgtcattccaaataaacctttggtaatcttcaacgattaccctaa

SEQ ID NO: 8 - protein, 695 aa, Homo sapiens
  source 1..695: note = amino acid sequence of protein AMPH NCBI Ref NP_001626.1; note (original language) = secuencia de aminoacidos de la proteína AMPH NCBI Ref NP_001626.1
MADIKTGIFAKNVQKRLNRAQEKVLQKLGKADETKDEQFEEYVQNFKRQEAEGTRLQRELRGYLAAIKGMQEASMKLTESLHEVYEPDWYGREDVKMVGEKCDVLWEDFHQKLVDGSLLTLDTYLGQFPDIKNRIAKRSRKLVDYDSARHHLEALQSSKRKDESRISKAEEEFQKAQKVFEEFNVDLQEELPSLWSRRVGFYVNTFKNVSSLEAKFHKEIAVLCHKLYEVMTKLGDQHADKAFTIQGAPSDSGPLRIAKTPSPPEEPSPLPSPTASPNHTLAPASPAPARPRSPSQTRKGPPVPPLPKVTPTKELQQENIISFFEDNFVPEISVTTPSQNEVPEVKKEETLLDLDFDPFKPEVTPAGSAGVTHSPMSQTLPWDLWTTSTDLVQPASGGSFNGFTQPQDTSLFTMQTDQSMICNLAESEQAPPTEPKAEEPLAAVTPAVGLDLGMDTRAEEPVEEAVIIPGADADAAVGTLVSAAEGAPGEEAEAEKATVPAGEGVSLEEAKIGTETTEGAESAQPEAEELEATVPQEKVIPSVVIEPASNHEEEGENEITIGAEPKETTEDAAPPGPTSETPELATEQKPIQDPQPTPSAPAMGAADQLASAREASQELPPGFLYKVETLHDFEAANSDELTLQRGDVVLVVPSDSEADQDAGWLVGVKESDWLQYRDLATYKGLFPENFTRRLD

SEQ ID NO: 9 - DNA, 6808 bp, Homo sapiens
  source 1..6808: mol_type = genomic DNA; note = nucleotide sequence of UNC5B gene NCBI Ref NM_001244889.2; note (original language) = secuencia de nucleotidos del gen UNC5B NCBI Ref NM_001244889.2
attgtggcaggcggctggggccggctagggcgccggagccgcacgcagccgcggggctccgagaggcgcgcactggggctgggactgcgcggcgccgccgctgcgagcgccactgagcggtcgcgcaacttcggaggcacagcgccggagccaggcgagcgctcagagacccggagccagaggggcgcgccggagcctcgttcgagagccggcgccaggcacccaccgcgctccgagtgccaggcggccctccgcgcagcgtggcttccgctgcccccacggaaggcacgggctggcgctgccgggcgccggggaggacggcgaggaggaggcggcggcggcggagacggcggcggcgagactggggccagggagacagccctgggggagaggcgcccgaaccaggccgcgggagcatgggggcccggagcggagctcggggcgcgctgctgctggcactgctgctctgctgggacccgaggctgagccaagcaggcactgattctggcagcgaggtgctccctgactccttcccgtcagcgccagcagagccgctgccctacttcctgcaggagccacaggacgcctacattgtgaagaacaagcctgtggagctccgctgccgcgccttccccgccacacagatctacttcaagtgcaacggcgagtgggtcagccagaacgaccacgtcacacaggaaggcctggatgaggccaccggcctgcgggtgcgcgaggtgcagatcgaggtgtcgcggcagcaggtggaggagctctttgggctggaggattactggtgccagtgcgtggcctggagctccgcgggcaccaccaagagtcgccgagcctacgtccgcatcgcctacctgcgcaagaacttcgatcaggagcctctgggcaaggaggtgcccctggaccatgaggttctcctgcagtgccgcccgccggagggggtgcctgtggccgaggtggaatggctcaagaatgaggatgtcatcgaccccacccaggacaccaacttcctgctcaccatcgaccacaacctcatcatccgccaggcccgcctgtcggacactgccaactatacctgcgtggccaagaacatcgtggccaaacgccggagcaccactgccaccgtcatcgtctacgtgaatggcggctggtccagctgggcagagtggtcaccctgctccaaccgctgtggccgaggctggcagaagcgcacccggacctgcaccaaccccgctccactcaacggaggggccttctgcgagggccaggcattccagaagaccgcctgcaccaccatctgcccagtcgatggggcgtggacggagtggagcaagtggtcagcctgcagcactgagtgtgcccactggcgtagccgcgagtgcatggcgcccccaccccagaacggaggccgtgactgcagcgggacgctgctcgactctaagaactgcacagatgggctgtgcatgcaaatgctggaggcctcaggggatgcggcgctgtatgcggggctcgtggtggccatcttcgtggtcgtggcaatcctcatggcggtgggggtggtggtgtaccgccgcaactgccgtgacttcgacacagacatcactgactcatctgctgccctgactggtggtttccaccccgtcaactttaagacggcaaggcccagcaacccgcagctcctacacccctctgtgcctcctgacctgacagccagcgccggcatctaccgcggacccgtgtatgccctgcaggactccaccgacaaaatccccatgaccaactctcctctgctggaccccttacccagccttaaggtcaaggtctacagctccagcaccacgggctctgggccaggcctggcagatggggctgacctgctgggggtcttgccgcctggcacataccctagcgatttcgcccgggacacccacttcctgcacctgcgcagcgccagcctcggttcccagcagctcttgggcctgccccgagacccagggagcagcgtcagcggcacctttggctgcctgggtgggaggctcagcatccccggcacaggggtcagcttgctggtgcccaatggagccattccccagggcaagttctacgagatgtatctactcatcaacaaggcagaaagtaccctcccgctttcagaagggacccagacagtattgagcccctcggtgacctgtggacccacaggcctcctgctgtgccgccccgtcatcctcaccatgccccactgtgccgaagtcagtgcccgtgactggatctttcagctcaagacccaggcccaccagggccactgggaggaggtggtgaccctggatgaggagaccctgaacacaccctgctactgccagctggagcccagggcctgtcacatcctgctggaccagctgggcacctacgtgttcacgggcgagtcctattcccgctcagcagtcaagcggctccagctggccgtcttcgcccccgccctctgcacctccctggagtacagcctccgggtctactgcctggaggacacgcctgtagcactgaaggaggtgctggagctggagcggactctgggcggatacttggtggaggagccgaaaccgctaatgttcaaggacagttaccacaacctgcgcctctccctccatgacctcccccatgcccattggaggagcaagctgctggccaaataccaggagatccccttctatcacatttggagtggcagccagaaggccctccactgcactttcaccctggagaggcacagcttggcctccacagagctcacctgcaagatctgcgtgcggcaagtggaaggggagggccagatattccagctgcataccactctggcagagacacctgctggctccctggacactctctgctctgcccctggcagcactgtcaccacccagctgggaccttatgccttcaagatcccactgtccatccgccagaagatatgcaacagcctagatgcccccaactcacggggcaatgactggcggatgttagcacagaagctctctatggaccggtacctgaattactttgccaccaaagcgagccccacgggtgtgatcctggacctctgggaagctctgcagcaggacgatggggacctcaacagcctggcgagtgccttggaggagatgggcaagagtgagatgctggtggctgtggccaccgacggggactgctgagcctcctgggacagcgggctggcagggactggcaggaggcaggtgcagggaggcctggggcagcctcctgatggggatgtttggcctctgcttcctcccagttcacagccagagttgcctctcctcctcctcttccccaacccccagaccatgaccagccttagaaaatccatgtactctgttgttagagggcccagagttccttctccacccccgctctctctctcttggcctgagatctctgtgcaggaaccaagatggggctgaagcctctggaggcagttggttgggggcgggcaggcaggaggccctccctccacccccccaccctcagcccggcaacttctgggttccatgggttttagttccgttctcgttttcttcctccgttattgatttctcctttctccctaagcccccttctgcttccacgcccttttcctctttgaagagtcaagtacaattcagacaaactgctttctcctgtccaaaagcaaaaaggcaaaggaaagaaagaaagcttcagaccgctagtaaggctcaaagaagaagaaaaacaccaaaaccacaagggaaaagaaaaacccagtttcttaggaaacgcaaacgatttattatccagattatttggataagtcctttttaagaaaaaaaaagaaaatgaaaaacaacacaaaaaaaatagaaaactcttttcttgagtgtggatgagaatgggcacgctcacacttctggccaggagtgaatgtgcctgtgtgtgtgtgtgtgtgtgtgtgtgtgtgtgtacatgtacgcgtgtgcattgaggagagagagactgaacagagagtactttgctgctaacgaatccatcttggactaaattctgacaaggcctcagtttccccagttgtgcagggagtaggtcagacagggttttcactgtctagatttagctggttagattttcctctaaaatcttaagcagatgctgaatccataaagccaaggagtgctgagggctggagtgggtgggccctccctcccacagccccagggagatacatctggactcctgggaatctggattaagaaagttgggatgaaagaggaggactgctcaggccagttgtgagccagggagaatgttccagtctggttttggtctggtggctcctagaaagggatgtggcccagaagtgggactcaaacagagagatgaagtaggggaggggagtcctccacgggcatctctctcctggcggctggatagctttaccctagggtggggccagccctgacaccctcatcccctcctcagcccagcagcctctagagcagcgtggtgctctcttgatggccaggaatccagaatctgcccttccccaaccttggtttctccttctgtaaagcagagtgatggctgagaagtcctctctagctgcagaagcctgagcttcccggtgtcagtcagctctgcaacgtgggagccttggaggcgggtggcctggctgtgcttcatatgcccaggagtggagaaggaggctgagaagctggtttcccagctctgatctccacaggcacctcctataaccctcctctcacccaccccgctacggtctgagagatctgaaataacctttcccagtgggcagggttgccagggttgaggggacagcacataccacccccacccaacctgttcgaggggccctgcatggcacgggatgagtccctgccctgtgcagctgcctggcagtggctgggacaaggatcttgcagccagcacagaggcctcttcaaaggcctctccctcttggcactccaggcaaggcaggtgcccgcttccccaacacctccaggcagtgaccctagggcatgccccagcaggtctccgagcagccactgggacccgtctcagcacatcctggcctttgaaagtctgatatcctgagaggagggcaggttttagggccgcagttccagccagcgtccccagcctggcttccctgccatggactcagtagctcgtggggcttcttaccacccaccagccccgctggggtgcggcctggctgtgggcaaaggaggacttgcctggagatttgagagaagattccttctaccagggctgctgaggggccaggcctgcatcaggggctaggctctggctgggcccggaggctgagactaaggctttcgaccctggtgcctccatgtggatgctgcctcagacaaaggcagtgagccttccctgccaaagtgcccatcccatgggctcggcctcactggtcactgttagcccatgaacacgtgtgggcctcggtcacgtggctttgagggcagtctgaccaggctagaccacacgtgccgtgacagggggtgccattcccctcgcaggctctaatgtgcccacatgtagcctggcagtccaaagaccaagaatcaacttgcaaatctgccattaaactgctgtgcgacttcaggcatatcactgccttctctgggcttcagtgtccttttcatacctagaagtctgcggtctgaggctctttgggttcagacacactgttctaggcttctgtaggggaccttgtgatctgccgtgcccctcctccctgttcttttctgtcctccccaccccaccctcagaagctgcttgctctgcccccaggacaggagcttgacggatgaagtgcagccagccacccaggtgccatttccagtctgacttccagaaatgtgcaccatgtcctagagcacagacccattggctggagcctcctgggagggttcaaaccatcagctctatgagaaatgcccagaaaggctttgccgactccatccgtctgtggaggctgcctgcctccggggtgggatgggtggtttctcctccaattcagacccaagaggtagcccccgagggcatgtacctggtgggaagcagctcaggtacccttgggggttgcagggcccttacgcaggtatttctctctctctcctctctggggtgcgtgtgtgcgtgcgcgtgtgcgtgcctatgcttttctctgtgggcacatcaggatgcccctcggagagcatgtgcacgtgtccccacctgagcgagcgtgtgtgtgtgctcctctgcgtcccaggtttggacgtctagggtttggtgtgcctgtcttctgccctccctgagcccacagggtcagtcaatgtatcttctacgtgcctctccctctgccttctctcacagtgcccccggctccagagctcaggggtaggggttctcctgagggtgcaggggatccttctcatctcctggaccctccagggcactctggtccctattccccagctcctaggcagctgagccgggtcccttaggggaggtgaccaggagctttggtgcagggagctcttggtggggcaaagggctggacccctgccaggtctgtggacatggttatatgcccgggagaggggggtgcagggccccagggatggcccccaatcccacctctgtttattctgtaaactgcaacctataaataacctttagcattcctattgtaacaaaattaatttttatgaaataaattatatttcctagtctaataaaa

SEQ ID NO: 10 - protein, 934 aa, Homo sapiens
  source 1..934: note = amino acid sequence of UNC5B protein NCBI Ref NP_001231818.1; note (original language) = secuencia de aminoacidos de la proteina UNC5B NCBI Ref NP_001231818.1
MGARSGARGALLLALLLCWDPRLSQAGTDSGSEVLPDSFPSAPAEPLPYFLQEPQDAYIVKNKPVELRCRAFPATQIYFKCNGEWVSQNDHVTQEGLDEATGLRVREVQIEVSRQQVEELFGLEDYWCQCVAWSSAGTTKSRRAYVRIAYLRKNFDQEPLGKEVPLDHEVLLQCRPPEGVPVAEVEWLKNEDVIDPTQDTNFLLTIDHNLIIRQARLSDTANYTCVAKNIVAKRRSTTATVIVYVNGGWSSWAEWSPCSNRCGRGWQKRTRTCTNPAPLNGGAFCEGQAFQKTACTTICPVDGAWTEWSKWSACSTECAHWRSRECMAPPPQNGGRDCSGTLLDSKNCTDGLCMQMLEASGDAALYAGLVVAIFVVVAILMAVGVVVYRRNCRDFDTDITDSSAALTGGFHPVNFKTARPSNPQLLHPSVPPDLTASAGIYRGPVYALQDSTDKIPMTNSPLLDPLPSLKVKVYSSSTTGSGPGLADGADLLGVLPPGTYPSDFARDTHFLHLRSASLGSQQLLGLPRDPGSSVSGTFGCLGGRLSIPGTGVSLLVPNGAIPQGKFYEMYLLINKAESTLPLSEGTQTVLSPSVTCGPTGLLLCRPVILTMPHCAEVSARDWIFQLKTQAHQGHWEEVVTLDEETLNTPCYCQLEPRACHILLDQLGTYVFTGESYSRSAVKRLQLAVFAPALCTSLEYSLRVYCLEDTPVALKEVLELERTLGGYLVEEPKPLMFKDSYHNLRLSLHDLPHAHWRSKLLAKYQEIPFYHIWSGSQKALHCTFTLERHSLASTELTCKICVRQVEGEGQIFQLHTTLAETPAGSLDTLCSAPGSTVTTQLGPYAFKIPLSIRQKICNSLDAPNSRGNDWRMLAQKLSMDRYLNYFATKASPTGVILDLWEALQQDDGDLNSLASALEEMGKSEMLVAVATDGDC

SEQ ID NO: 11 - DNA, 2039 bp, Homo sapiens
  source 1..2039: mol_type = genomic DNA; note = nucleotide sequence of OAT gene NCBI Ref NM_000274.4; note (original language) = secuencia de nucleotidos del gen OAT NCBI Ref NM_000274.4
gttgcgcttcatagacgccgcgtgtacccggttgtcctcaggcgctgtcagatctgtggtttttctacttgaaggacacaatgttttccaaactagcacatttgcagaggtttgctgtacttagtcgcggagttcattcttcagtggcttctgctacatctgttgcaactaaaaaaacagtccaaggccctccaacctctgatgacatttttgaaagggaatataagtatggtgcacacaactaccatcctttacctgtagccctggagagaggaaaaggtatttacttatgggatgtagaaggcagaaaatattttgacttcctgagttcttacagtgctgtcaaccaagggcattgtcaccccaagattgtgaatgctctgaagagtcaagtggacaaattgaccttaacatctagagctttctataataacgtacttggtgaatatgaggagtatattactaaacttttcaactaccacaaagttcttcctatgaatacaggagtggaggctggagagactgcctgtaaactagctcgtaagtggggctataccgtgaagggcattcagaaatacaaagcaaagattgtttttgcagctgggaacttctggggtaggacgttgtctgctatctccagttccacagacccaaccagttacgatggttttggaccatttatgccgggattcgacatcattccctataatgatctgcccgcactggagcgtgctcttcaggatccaaatgtggctgcgttcatggtagaaccaattcagggtgaagcaggcgttgttgttccggatccaggttacctaatgggagtgcgagagctctgcaccaggcaccaggttctctttattgctgatgaaatacagacaggattggccagaactggtagatggctggctgttgattatgaaaatgtcagacctgatatagtcctccttggaaaggccctttctgggggcttataccctgtgtctgcagtgctgtgtgatgatgacatcatgctgaccattaagccaggggagcatgggtccacatacggtggcaatccactaggctgccgagtggccatcgcagcccttgaggttttagaagaagaaaaccttgctgaaaatgcagacaaattgggcattatcttgagaaatgaactcatgaagctaccttctgatgttgtaactgccgtaagaggaaaaggattattaaacgctattgtcattaaagaaaccaaagattgggatgcttggaaggtgtgtctacgacttcgagataatggacttctggccaagccaacccatggcgacattatcaggtttgcgcctccgctggtgatcaaggaggatgagcttcgagagtccattgaaattattaacaagaccatcttgtctttctgagggtagccagctgttttcagtggtccctgggagccagctggagacaggtggtcctgtaaaagctttattcctaatgtgggcacattccactcccatgagtcttcaaaaactttttttttgaatatatttttttcagttgatacataatagaacaacgtttatgaacctgccgtttgctttgtaacgtaactaaataatgtaatggcatctatattcagttgaagtgttttgatgtgcatgtgtacttcctaaggtgaaatgcatctatatacagacagcctctaaatcaagtccttcagtataattgatatatgtttttataatttcctcactggtataagtgtttcatatttgaaaaagttatctctgggtattgcataaaaggcttcatcttataaagtgaaatcattgttattgaattttaggaaggattaatggttaagtgtatataaaatactaatattaagtaaacttcatattggccaacaccagggttgtattctatggatgtcattattttgaattaagaattagtgtttaacattcctaaattgttttgagtgcttgattataatttgtaaaaaatgtttattttcaatacttctttaaatttaaaataaagcttatatttcaaatgtc

SEQ ID NO: 12 - protein, 439 aa, Homo sapiens
  source 1..439: note = amino acid sequence of OAT protein NCBI Ref NP_000265.1; note (original language) = secuencia de aminoacidos de la proteina OAT NCBI Ref NP_000265.1
MFSKLAHLQRFAVLSRGVHSSVASATSVATKKTVQGPPTSDDIFEREYKYGAHNYHPLPVALERGKGIYLWDVEGRKYFDFLSSYSAVNQGHCHPKIVNALKSQVDKLTLTSRAFYNNVLGEYEEYITKLFNYHKVLPMNTGVEAGETACKLARKWGYTVKGIQKYKAKIVFAAGNFWGRTLSAISSSTDPTSYDGFGPFMPGFDIIPYNDLPALERALQDPNVAAFMVEPIQGEAGVVVPDPGYLMGVRELCTRHQVLFIADEIQTGLARTGRWLAVDYENVRPDIVLLGKALSGGLYPVSAVLCDDDIMLTIKPGEHGSTYGGNPLGCRVAIAALEVLEEENLAENADKLGIILRNELMKLPSDVVTAVRGKGLLNAIVIKETKDWDAWKVCLRLRDNGLLAKPTHGDIIRFAPPLVIKEDELRESIEIINKTILSF

SEQ ID NO: 13 - DNA, 3052 bp, Homo sapiens
  source 1..3052: mol_type = genomic DNA; note = nucleotide sequence of EZR gene NCBI Ref NM_001111077.2; note (original language) = secuencia de nucleotidos del gen EZR NCBI Ref NM_001111077.2
actcggcggacgcaagggcggcggggagcacacggagcactgcaggcgccgggttgggacagcgtcttcgctgctgctggatagtcgtgttttcggggatcgaggatactcaccagaaaccgaaaatgccgaaaccaatcaatgtccgagttaccaccatggatgcagagctggagtttgcaatccagccaaatacaactggaaaacagctttttgatcaggtggtaaagactatcggcctccgggaagtgtggtactttggcctccactatgtggataataaaggatttcctacctggctgaagctggataagaaggtgtctgcccaggaggtcaggaaggagaatcccctccagttcaagttccgggccaagttctaccctgaagatgtggctgaggagctcatccaggacatcacccagaaacttttcttcctccaagtgaaggaaggaatccttagcgatgagatctactgcccccctgagactgccgtgctcttggggtcctacgctgtgcaggccaagtttggggactacaacaaagaagtgcacaagtctgggtacctcagctctgagcggctgatccctcaaagagtgatggaccagcacaaacttaccagggaccagtgggaggaccggatccaggtgtggcatgcggaacaccgtgggatgctcaaagataatgctatgttggaatacctgaagattgctcaggacctggaaatgtatggaatcaactatttcgagataaaaaacaagaaaggaacagacctttggcttggagttgatgcccttggactgaatatttatgagaaagatgataagttaaccccaaagattggctttccttggagtgaaatcaggaacatctctttcaatgacaaaaagtttgtcattaaacccatcgacaagaaggcacctgactttgtgttttatgccccacgtctgagaatcaacaagcggatcctgcagctctgcatgggcaaccatgagttgtatatgcgccgcaggaagcctgacaccatcgaggtgcagcagatgaaggcccaggcccgggaggagaagcatcagaagcagctggagcggcaacagctggaaacagagaagaaaaggagagaaaccgtggagagagagaaagagcagatgatgcgcgagaaggaggagttgatgctgcggctgcaggactatgaggagaagacaaagaaggcagagagagagctctcggagcagattcagagggccctgcagctggaggaggagaggaagcgggcacaggaggaggccgagcgcctagaggctgaccgtatggctgcactgcgggctaaggaggagctggagagacaggcggtggatcagataaagagccaggagcagctggctgcggagcttgcagaatacactgccaagattgccctcctggaagaggcgcggaggcgcaaggaggatgaagttgaagagtggcagcacagggccaaagaagcccaggatgacctggtgaagaccaaggaggagctgcacctggtgatgacagcacccccgcccccaccaccccccgtgtacgagccggtgagctaccatgtccaggagagcttgcaggatgagggcgcagagcccacgggctacagcgcggagctgtctagtgagggcatccgggatgaccgcaatgaggagaagcgcatcactgaggcagagaagaacgagcgtgtgcagcggcagctgctgacgctgagcagcgagctgtcccaggcccgagatgagaataagaggacccacaatgacatcatccacaacgagaacatgaggcaaggccgggacaagtacaagacgctgcggcagatccggcagggcaacaccaagcagcgcatcgacgagttcgaggccctgtaacagccaggccaggaccaagggcagaggggtgctcatagcgggcgctgccagccccgccacgcttgtgtctttagtgctccaagtctaggaactccctcagatcccagttcctttagaaagcagttacccaacagaaacattctgggctgggaaccagggaggcgccctggtttgttttccccagttgtaatagtgccaagcaggcctgattctcgcgattattctcgaatcacctcctgtgttgtgctgggagcaggactgattgaattacggaaaatgcctgtaaagtctgagtaagaaacttcatgctggcctgtgtgatacaagagtcagcatcattaaaggaaacgtggcaggacttccatctgtgccatacttgttctgtattcgaaatgagctcaaattgattttttaatttctatgaaggatccatctttgtatatttacatgcttagaggggtgaaaattattttggaaattgagtctgaagcactctcgcacacacagtgattccctcctcccgtcactccacgcagctggcagagagcacagtgatcaccagcgtgagtggtggaggaggacacttggatttttttttttgttttttttttttttgcttaacagttttagaatacattgtacttatacaccttattaatgatcagctatatactatttatatacaagtgataatacagatttgtaacattagttttaaaaagggaaagttttgttctgtatattttgttaccttttacagaataaaagaattacatatgaaaaaccctctaaaccatggcacttgatgtgatgtggcaggagggcagtggtggagctggacctgcctgctgcagtcacgtgtaaacaggattattattagtgttttatgcatgtaatggactatgcacacttttaattttgtcagattcacacatgccactatgagctttcagactccagctgtgaagagactctgtttgcttgtgtttgtttgtttgcagtctctctctgccatggccttggcaggctgctggaaggcagcttgtggaggccgttggttccgcccactcattccttctcgtgcactgctttctccttcacagctaagatgccatgtgcaggtggattccatgccgcagacatgaaataaaagctttgcaaaggca

SEQ ID NO: 14 - protein, 586 aa, Homo sapiens
  source 1..586: note = amino acid sequence of EZR protein NCBI Ref NP_001104547.1; note (original language) = secuencia de aminoacidos de la proteina EZR NCBI Ref NP_001104547.1
MPKPINVRVTTMDAELEFAIQPNTTGKQLFDQVVKTIGLREVWYFGLHYVDNKGFPTWLKLDKKVSAQEVRKENPLQFKFRAKFYPEDVAEELIQDITQKLFFLQVKEGILSDEIYCPPETAVLLGSYAVQAKFGDYNKEVHKSGYLSSERLIPQRVMDQHKLTRDQWEDRIQVWHAEHRGMLKDNAMLEYLKIAQDLEMYGINYFEIKNKKGTDLWLGVDALGLNIYEKDDKLTPKIGFPWSEIRNISFNDKKFVIKPIDKKAPDFVFYAPRLRINKRILQLCMGNHELYMRRRKPDTIEVQQMKAQAREEKHQKQLERQQLETEKKRRETVEREKEQMMREKEELMLRLQDYEEKTKKAERELSEQIQRALQLEEERKRAQEEAERLEADRMAALRAKEELERQAVDQIKSQEQLAAELAEYTAKIALLEEARRRKEDEVEEWQHRAKEAQDDLVKTKEELHLVMTAPPPPPPPVYEPVSYHVQESLQDEGAEPTGYSAELSSEGIRDDRNEEKRITEAEKNERVQRQLLTLSSELSQARDENKRTHNDIIHNENMRQGRDKYKTLRQIRQGNTKQRIDEFEAL

SEQ ID NO: 15 - DNA, 3472 bp, Homo sapiens
  source 1..3472: mol_type = genomic DNA; note = nucleotide sequence of NR4A2 gene NCBI Ref NM_006186.4; note (original language) = secuencia de nucleotidos del gen NR4A2 NCBI Ref NM_006186.4
aagccacataaacaaaggcacattggcggccagggccagtccgcccggcggctcgcgcacggctccgcggtcccttttgcctgtccagccggccgcctgtccctgctccctccctccgtgaggtgtccgggttcccttcgcccagctctcccacccctacccgaccccggcgcccgggctcccagagggaactgcacttcggcagagttgaatgaatgaagacagacgcggagaactcctaaggaggagattggacaggctggactccccattgcttttctaaaaatcttggaaactttgtccttcattgaattacgacactgtccacctttaatttcctcgaaaacgcctgtaactcggctgaagccatgccttgtgttcaggcgcagtatgggtcctcgcctcaaggagccagccccgcttctcagagctacagttaccactcttcgggagaatacagctccgatttcttaactccagagtttgtcaagtttagcatggacctcaccaacactgaaatcactgccaccacttctctccccagcttcagtacctttatggacaactacagcacaggctacgacgtcaagccaccttgcttgtaccaaatgcccctgtccggacagcagtcctccattaaggtagaagacattcagatgcacaactaccagcaacacagccacctgcccccccagtctgaggagatgatgccgcactccgggtcggtttactacaagccctcctcgcccccgacgcccaccaccccgggcttccaggtgcagcacagccccatgtgggacgacccgggatctctccacaacttccaccagaactacgtggccactacgcacatgatcgagcagaggaaaacgccagtctcccgcctctccctcttctcctttaagcaatcgccccctggcaccccggtgtctagttgccagatgcgcttcgacgggcccctgcacgtccccatgaacccggagcccgccggcagccaccacgtggtggacgggcagaccttcgctgtgcccaaccccattcgcaagcccgcgtccatgggcttcccgggcctgcagatcggccacgcgtctcagctgctcgacacgcaggtgccctcaccgccgtcgcggggctccccctccaacgaggggctgtgcgctgtgtgtggggacaacgcggcctgccaacactacggcgtgcgcacctgtgagggctgcaaaggcttctttaagcgcacagtgcaaaaaaatgcaaaatacgtgtgtttagcaaataaaaactgcccagtggacaagcgtcgccggaatcgctgtcagtactgccgatttcagaagtgcctggctgttgggatggtcaaagaagtggttcgcacagacagtttaaaaggccggagaggtcgtttgccctcgaaaccgaagagcccacaggagccctctcccccttcgcccccggtgagtctgatcagtgccctcgtcagggcccatgtcgactccaacccggctatgaccagcctggactattccaggttccaggcgaaccctgactatcaaatgagtggagatgacacccagcatatccagcaattctatgatctcctgactggctccatggagatcatccggggctgggcagagaagatccctggcttcgcagacctgcccaaagccgaccaagacctgctttttgaatcagctttcttagaactgtttgtccttcgattagcatacaggtccaacccagtggagggtaaactcatcttttgcaatggggtggtcttgcacaggttgcaatgcgttcgtggctttggggaatggattgattccattgttgaattctcctccaacttgcagaatatgaacatcgacatttctgccttctcctgcattgctgccctggctatggtcacagagagacacgggctcaaggaacccaagagagtggaagaactgcaaaacaagattgtaaattgtctcaaagaccacgtgactttcaacaatggggggttgaaccgccccaattatttgtccaaactgttggggaagctcccagaacttcgtaccctttgcacacaggggctacagcgcattttctacctgaaattggaagacttggtgccaccgccagcaataattgacaaacttttcctggacactttacctttctaagacctcctcccaagcacttcaaaggaactggaatgataatggaaactgtcaagagggggcaagtcacatgggcagagatagccgtgtgagcagtctcagctcaagctgccccccatttctgtaaccctcctagcccccttgatccctaaagaaaacaaacaaacaaacaaaaactgttgctatttcctaacctgcaggcagaacctgaaagggcattttggctccggggcatcctggatttagaacatggactacacacaatacagtggtataaactttttattctcagtttaaaaatcagtttgttgttcagaagaaagattgctataatgtataatgggaaatgtttggccatgcttggttgttgcagttcagacaaatgtaacacacacacacatacacacacacacacacacacagagacacatcttaaggggacccacaagtattgccctttaacaagacttcaaagttttctgctgtaaagaaagctgtaatatatagtaaaactaaatgttgcgtgggtggcatgagttgaagaaggcaaaggcttgtaaatttacccaatgcagtttggctttttaaattattttgtgcctatttatgaataaatattacaaattctaaaagataagtgtgtttgcaaaaaaaaagaaaataaatacataaaaaagggacaagcatgttgattctaggttgaaaatgttataggcacttgctacttcagtaatgtctatattatataaatagtatttcagacactatgtagtctgttagattttataaagattggtagttatctgagcttaaacattttctcaattgtaaaataggtgggcacaagtattacacatcagaaaatcctgacaaaagggacacatagtgtttgtaacaccgtccaacattccttgtttgtaagtgttgtatgtaccgttgatgttgataaaaagaaagtttatatcttgattattttgttgtctaaagctaaacaaaacttgcatgcagcagcttttgactgtttccagagtgcttataatatacataactccctggaaataactgagcactttgaattttttttatgtctaaaattgtcagttaatttattattttgtttgagtaagaattttaatattgccatattctgtagtatttttctttgtatatttctagtatggcacatgatatgagtcactgcctttttttctatggtgtatgacagttagagatgctgattttttttctgataaattctttctttgagaaagacaattttaatgtttacaacaataaaccatgtaaatgaa

SEQ ID NO: 16 - protein, 598 aa, Homo sapiens
  source 1..598: note = amino acid sequence of NR4A2 protein NCBI Ref NP_006177.1; note (original language) = secuencia de aminoacidos de la proteina NR4A2 NCBI Ref NP_006177.1
MPCVQAQYGSSPQGASPASQSYSYHSSGEYSSDFLTPEFVKFSMDLTNTEITATTSLPSFSTFMDNYSTGYDVKPPCLYQMPLSGQQSSIKVEDIQMHNYQQHSHLPPQSEEMMPHSGSVYYKPSSPPTPTTPGFQVQHSPMWDDPGSLHNFHQNYVATTHMIEQRKTPVSRLSLFSFKQSPPGTPVSSCQMRFDGPLHVPMNPEPAGSHHVVDGQTFAVPNPIRKPASMGFPGLQIGHASQLLDTQVPSPPSRGSPSNEGLCAVCGDNAACQHYGVRTCEGCKGFFKRTVQKNAKYVCLANKNCPVDKRRRNRCQYCRFQKCLAVGMVKEVVRTDSLKGRRGRLPSKPKSPQEPSPPSPPVSLISALVRAHVDSNPAMTSLDYSRFQANPDYQMSGDDTQHIQQFYDLLTGSMEIIRGWAEKIPGFADLPKADQDLLFESAFLELFVLRLAYRSNPVEGKLIFCNGVVLHRLQCVRGFGEWIDSIVEFSSNLQNMNIDISAFSCIAALAMVTERHGLKEPKRVEELQNKIVNCLKDHVTFNNGGLNRPNYLSKLLGKLPELRTLCTQGLQRIFYLKLEDLVPPPAIIDKLFLDTLPF

SEQ ID NO: 17 - DNA, 22 bp, synthetic construct
  source 1..22: mol_type = other DNA; note = NR4A2 forward primer sequence; note (original language) = NR4A2 secuencia del cebador directo; organism (original language) = construccion sintetica
gactatcaaatgagtggagatg

SEQ ID NO: 18 - DNA, 20 bp, synthetic construct
  source 1..20: mol_type = other DNA; note = NR4A2 reverse primer sequence; note (original language) = NR4A2 secuencia del cebador reverso; organism (original language) = construccion sintetica
gacctgtatgctaatcgaag

SEQ ID NO: 19 - DNA, 20 bp, synthetic construct
  source 1..20: mol_type = other DNA; note = OAT forward primer sequence; note (original language) = OAT secuencia del cebador directo; organism (original language) = construccion sintetica
cagacctgatatagtcctcc

SEQ ID NO: 20 - DNA, 21 bp, synthetic construct
  source 1..21: mol_type = other DNA; note = OAT reverse primer sequence; note (original language) = OAT secuencia del cebador reverso; organism (original language) = construccion sintetica
cttcttctaaaacctcaaggg

SEQ ID NO: 21 - DNA, 21 bp, synthetic construct
  source 1..21: mol_type = other DNA; note = AMPH forward primer sequence; note (original language) = AMPH secuencia del cebador directo; organism (original language) = construccion sintetica
cctgacataaagaatcgcatc

SEQ ID NO: 22 - DNA, 20 bp, synthetic construct
  source 1..20: mol_type = other DNA; note = AMPH reverse primer sequence; note (original language) = AMPH secuencia del cebador reverso; organism (original language) = construccion sintetica
caaacactttctgtgctttc

SEQ ID NO: 23 - DNA, 18 bp, synthetic construct
  source 1..18: mol_type = other DNA; note = NUDT2 forward primer sequence; note (original language) = NUDT2 secuencia del cebador directo; organism (original language) = construccion sintetica
ttctgcttcggtccttag

SEQ ID NO: 24 - DNA, 20 bp, synthetic construct
  source 1..20: mol_type = other DNA; note = NUDT2 reverse primer sequence; note (original language) = NUDT2 secuencia del cebador reverso; organism (original language) = construccion sintetica
aactcaattgcattgttgtc

SEQ ID NO: 25 - DNA, 18 bp, synthetic construct
  source 1..18: mol_type = other DNA; note = UNC5B forward primer sequence; note (original language) = UNC5B secuencia del cebador directo; organism (original language) = construccion sintetica
aggacagttaccacaacc

SEQ ID NO: 26 - DNA, 19 bp, synthetic construct
  source 1..19: mol_type = other DNA; note = UNC5B reverse primer sequence; note (original language) = UNC5B secuencia del cebador reverso; organism (original language) = construccion sintetica
ggggatctcctggtatttg

SEQ ID NO: 27 - DNA, 20 bp, synthetic construct
  source 1..20: mol_type = other DNA; note = EZR forward primer sequence; note (original language) = EZR secuencia del cebador directo; organism (original language) = construccion sintetica
tgactttgtgttttatgccc

SEQ ID NO: 28 - DNA, 21 bp, synthetic construct
  source 1..21: mol_type = other DNA; note = EZR reverse primer sequence; note (original language) = EZR secuencia del cebador reverso; organism (original language) = construccion sintetica
ctccttttcttctctgtttcc

SEQ ID NO: 29 - DNA, 18 bp, synthetic construct
  source 1..18: mol_type = other DNA; note = GAPDH forward primer sequence; note (original language) = GAPDH secuencia del cebador directo; organism (original language) = construccion sintetica
acagttgccatgtagacc

SEQ ID NO: 30 - DNA, 19 bp, synthetic construct
  source 1..19: mol_type = other DNA; note = GAPDH reverse primer sequence; note (original language) = GAPDH secuencia del cebador reverso; organism (original language) = construccion sintetica
ttgagcacagggtacttta

SEQ ID NO: 31 - DNA, 20 bp, synthetic construct
  source 1..20: mol_type = other DNA; note = Actb forward primer sequence; note (original language) = actb secuencia del cebador directo; organism (original language) = construccion sintetica
gatgtatgaaggctttggtc

SEQ ID NO: 32 - DNA, 20 bp, synthetic construct
  source 1..20: mol_type = other DNA; note = actb reverse primer sequence; note (original language) = actb secuencia del cebador reverso; organism (original language) = construccion sintetica
tgtgcacttttattggtctc

SEQ ID NO: 33 - DNA, 25 bp, synthetic construct
  source 1..25: mol_type = other DNA; note = GFP forward primer sequence; note (original language) = GFP secuencia del cebador directo; organism (original language) = construccion sintetica
caacagccacaacgtctatatcatg

SEQ ID NO: 34 - DNA, 21 bp, synthetic construct
  source 1..21: mol_type = other DNA; note = GFP reverse primer sequence; note (original language) = GFP secuencia del cebador reverso; organism (original language) = construccion sintetica
atgttgtggcggatcttgaag

SEQ ID NO: 35 - DNA, 19 bp, synthetic construct
  source 1..19: mol_type = other DNA; note = Rim forward primer sequence; note (original language) = Rim secuencia del cebador directo; organism (original language) = construccion sintetica
cagcaacagcccagatcag

SEQ ID NO: 36 - DNA, 20 bp, synthetic construct
  source 1..20: mol_type = other DNA; note = Rim reverse primer sequence; note (original language) = Rim secuencia del cebador reverso; organism (original language) = construccion sintetica
ctcatcaggccatcgagttc

SEQ ID NO: 37 - DNA, 20 bp, synthetic construct
  source 1..20: mol_type = other DNA; note = Rut forward primer sequence; note (original language) = Rut secuencia del cebador directo; organism (original language) = construccion sintetica
gaaacgttcaggtgtcggag

SEQ ID NO: 38 - DNA, 20 bp, synthetic construct
  source 1..20: mol_type = other DNA; note = Rut reverse primer sequence; note (original language) = Rut secuencia del cebador reverso; organism (original language) = construccion sintetica
cgattcgttggctgatggtg

SEQ ID NO: 39 - DNA, 20 bp, synthetic construct
  source 1..20: mol_type = other DNA; note = dnc forward primer sequence; note (original language) = dnc secuencia del cebador directo; organism (original language) = construccion sintetica
caaacgcatgctcaacaagg

SEQ ID NO: 40 - DNA, 20 bp, synthetic construct
  source 1..20: mol_type = other DNA; note = dnc reverse primer sequence; note (original language) = dnc secuencia del cebador reverso; organism (original language) = construccion sintetica
gatggcaagtcgaactcctg

SEQ ID NO: 41 - DNA, 20 bp, synthetic construct
  source 1..20: mol_type = other DNA; note = amn forward primer sequence; note (original language) = amn secuencia del cebador directo; organism (original language) = construccion sintetica
caaatgttccgagcgtccac

SEQ ID NO: 42 - DNA, 20 bp, synthetic construct
  source 1..20: mol_type = other DNA; note = amn reverse primer sequence; note (original language) = amn secuencia del cebador reverso; organism (original language) = construccion sintetica
gcagcggttccgtttgatac

SEQ ID NO: 43 - DNA, 22 bp, synthetic construct
  source 1..22: mol_type = other DNA; note = CaMKII forward primer sequence; note (original language) = CaMKII secuencia del cebador directo; organism (original language) = construccion sintetica
gggagccatacttacgacaatg

SEQ ID NO: 44 - DNA, 22 bp, synthetic construct
  source 1..22: mol_type = other DNA; note = CaMKII reverse primer sequence; note (original language) = CaMKII secuencia del cebador reverso; organism (original language) = construccion sintetica
tcggttgattctttgacctgtg

SEQ ID NO: 45 - DNA, 20 bp, synthetic construct
  source 1..20: mol_type = other DNA; note = Orb2 forward primer sequence; note (original language) = Orb2 secuencia del cebador directo; organism (original language) = construccion sinteteica
aactgtgactccctctccag

SEQ ID NO: 46 - DNA, 20 bp, synthetic construct
  source 1..20: mol_type = other DNA; note = Orb2 reverse primer sequence; note (original language) = Orb2 secuencia del cebador reverso; organism (original language) = construccion sintetica
ttgcgcagactaacttcgtc

SEQ ID NO: 47 - DNA, 20 bp, synthetic construct
  source 1..20: mol_type = other DNA; note = 1tub23cf forward primer sequence; note (original language) = 1tub23cf secuencia del cebador directo; organism (original language) = construccion sintetica
taatgggctcggtctactcc

SEQ ID NO: 48 - DNA, 19 bp, synthetic construct
  source 1..19: mol_type = other DNA; note = 1tub23cf reverse primer sequence and RNApol2_Q forward primer sequence; note (original language) = 1tub23cf secuencia del cebador reverso y RNApol2_Q secuencia de cebador directo; organism (original language) = construccion sintetica
ccgcgatacttctctccac

SEQ ID NO: 49 - DNA, 19 bp, synthetic construct
  source 1..19: mol_type = other DNA; note = RNApol2_Q reverse primer sequence; note (original language) = RNApol2_Q secuencia del cebador reverso; organism (original language) = construccion sintetica
gaccagctaggcgacattc